European Patent Application EP 4 219 723 A1, published August 2, 2023. Title: CIRCULAR RNA PLATFORMS, USES THEREOF, AND THEIR MANUFACTURING PROCESSES FROM ENGINEERED DNA. Applicant: SYTE.bio. Application US 63279801, filed November 16, 2021. The sequence listing filed with the application follows.

SEQUENCE LISTING (12 sequences)

SEQ ID NO: 1 - DNA, 3045 bp, synthetic construct
  source 1..3045: mol_type = other DNA
  misc_feature 1..3045: function = circRNA transcription template plasmid DNA
gtccgttgtttatttttctaaatacattcaaatatgtatccgctcatgagacaataaccctgataaatgcttcaataatattgaaaaaggaagagtatgagtattcaacatttccgtgtcgcccttattcccttttttgcggcattttgccttcctgtttttgctcacccagaaacgctggtgaaagtaaaagatgctgaagatcagttgggtgcacgagtgggttacatcgaactggatctcaacagcggtaagatccttgagagttttcgccccgaagaacgtttcccaatgatgagcacttttaaagttctgctatgtggcgcggtattatcccgtgttgacgccgggcaagagcaactcggtcgccgcatacactattctcagaatgacttggttgagtactcaccagtcacagaaaagcatcttacggatggcatgacagtaagagaattatgcagtgctgccataaccatgagtgataacactgcggccaacttacttctgacaacgatcggaggaccgaaggagctaaccgcttttttgcacaacatgggggatcatgtaactcgccttgatcgttgggaaccggagctgaatgaagccataccaaacgacgagcgtgacaccacgatgcctgtagcaatggcaacaacgttgcgcaaactattaactggcgaactacttactctagcttcccggcaacaattaatagactggatggaggcggataaagttgcaggaccacttctgcgctcggcccttccggctggctggtttattgctgataaatctggagccggtgagcgtgggtctcgcggtatcattgcagcactggggccagatggtaagccctcccgtatcgtagttatctacacgacggggagtcaggcaactatggatgaacgaaatagacagatcgctgagataggtgcctcactgattaagcattggtaactgtcagaccaagtttactcatatatactttagattgatttccttaggactgagcgtcaaccccgtagaaaagatcaaaggatcttcttgagatcctttttttctgcgcgtaatctgctgcttgcaaacaaaaaaaccaccgctaccagcggtggtttgtttgccggatcaagagctaccaactctttttccgaaggtaactggcttcagcagagcgcagataccaaatactgtccttctagtgtagccgtagttaggccaccacttcaagaactctgtagcaccgcctacatacctcgctctgctaatcctgttaccagtggctgctgccagtggcgataagtcgtgtcttaccgggttggactcaagacgatagttaccggataaggcgcagcggtcgggctgaacggggggttcgtgcacacagcccagcttggagcgaacgacctacaccgaactgagatacctacagcgtgagctatgagaaagcgccacgcttcccgaagggagaaaggcggacaggtatccggtaagcggcagggtcggaacaggagagcgcacgagggagcttccagggggaaacgcctggtatctttatagtcctgtcgggtttcgccacctctgacttgagcgtcgatttttgtgatgctcgtcaggggggcggagcctatggaaaaacgccagcaacgcggcctttttacggttcctggccttttgctggccttttgctcacgaattaattcatgagcggatacatatttgaatgtatttagaaaaataaacaaataggggttccgcgcacatttccccgaataatacgactcactataggnnnnnnnnnnnnnnnnnnnnnnnnnnnnnnnnnnnnnnnnaacaacagataacttacagctatcggaaggtgcagagactcgacgggagctaccctaacgtcaagacgagggtaaagatgagagtccaattctcaaagccaataggcagtagcgaaagctgcgggagaagaaaatccgttgaccttaaacggtcgtgtgggttcaagtccctccacccccannnnnnnnnnnnnnnnnnnnnnnnnnnnnnnnnnnnnnnncccgggtctagaaaacgcaatagcggaaaaactttaaacattaaaacccccctctccctccccccctaacgttactggccgaagccgcttggaataaggccggtgtgcgtttgtctatatgttattttccaccatattgccgtcttttggcaatgtgagggcccggaaacctggccctgtcttcttgacgagcattcctaggggtctttcccctctcgccaaaggaatgcaaggtctgttgaatgtcgtgaaggaagcagttcctctggaagcttcttgaagacaaacaacgtctgtagcgaccctttgcaggcagcggaaccccccacctggcgacaggtgcctctgcggccaaaagccacgtgtataagatacacctgcaaaggcggcacaaccccagtgccacgttgtgagttggatagttgtggaaagagtcaaatggctctcctcaagcgtattcaacaaggggctgaaggatgcccagaaggtaccccattgtatgggatctgatctggggcctcggtgcacatgctttacatgtgtttagtcgaggttaaaaaacgtctaggccccccgaaccacggggacgtggttttcctttgaaaaacacgatgataatatggccacaaccatggagacgctgtccatggtgagagatctgtagctcgagctgtaatttacaaaaaacaaaacggcttaaatgcctaannnnnnnnnnnnnnnnnnnnnnnnnnnnnnnnnnnnnnnntgaagagaaaagcaagttcttgtaagtttaaccataaatttgccagccacggcaagctagacgctacggacttaaataattgagccttagagaagaaattctttaagtggatactctcaaactcagggaaacctaaatctagcgatagacaaggcaatcctgagccaagccgaagtagtaattagtaagttnnnnnnnnnnnnnnnnnnnnnnnnnnnnnnnnnnnnnnnnataacagcatatctag

SEQ ID NO: 2 - DNA, 17 bp, synthetic construct
  source 1..17: mol_type = other DNA
ggacaagatcgcgcgga

SEQ ID NO: 3 - DNA, 17 bp, synthetic construct
  source 1..17: mol_type = other DNA
agtgcacgagtctcagg

SEQ ID NO: 4 - DNA, 17 bp, synthetic construct
  source 1..17: mol_type = other DNA
cctgttctagcgcgcct

SEQ ID NO: 5 - DNA, 17 bp, synthetic construct
  source 1..17: mol_type = other DNA
tcacgtgctcagagtcc

SEQ ID NO: 6 - DNA, 17 bp, synthetic construct
  source 1..17: mol_type = other DNA
ggactctgagcacgtga

SEQ ID NO: 7 - DNA, 17 bp, synthetic construct
  source 1..17: mol_type = other DNA
ggacaagatcgcgcgga

SEQ ID NO: 8 - DNA, 74 bp, synthetic construct
  source 1..74: mol_type = other DNA
  misc_feature 1..74: function = SYTE-DNAzRL12 deoxyribozyme
nnnnnnnnnnnnnntccgcttgataccgagcgtcggcaatgccgtgttgattgatgatccnnnnnnnnnnnnnn

SEQ ID NO: 9 - DNA, 67 bp, synthetic construct
  source 1..67: mol_type = other DNA
  misc_feature 1..67: function = SYTE-DNAzRL16 deoxyribozyme
nnnnnnnnnnnnnnggatgcatacatcgctgcgcatagcgcagtacatacaacnnnnnnnnnnnnnn

SEQ ID NO: 10 - DNA, 261 bp, synthetic construct
  source 1..261: mol_type = other DNA
  misc_feature 1..261: function = pSYTEcRNA circularization sequence 1
nnnnnnnnnnnnnnnnnnnnnnnnnnnnnnnnnnnnnnnnaacaacagataacttacagctatcggaaggtgcagagactcgacgggagctaccctaacgtcaagacgagggtaaagatgagagtccaattctcaaagccaataggcagtagcgaaagctgcgggagaagaaaatccgttgaccttaaacggtcgtgtgggttcaagtccctccacccccannnnnnnnnnnnnnnnnnnnnnnnnnnnnnnnnnnnnnnn

SEQ ID NO: 11 - DNA, 271 bp, synthetic construct
  source 1..271: mol_type = other DNA
  misc_feature 1..271: function = pSYTEcRNA circularization sequence 2
nnnnnnnnnnnnnnnnnnnnnnnnnnnnnnnnnnnnnnnntgaagagaaaagcaagttcttgtaagtttaaccataaatttgccagccacggcaagctagacgctacggacttaaataattgagccttagagaagaaattctttaagtggatactctcaaactcagggaaacctaaatctagcgatagacaaggcaatcctgagccaagccgaagtagtaattagtaagttnnnnnnnnnnnnnnnnnnnnnnnnnnnnnnnnnnnnnnnn

SEQ ID NO: 12 - RNA, 1574 nt, synthetic construct
  source 1..1574: mol_type = other RNA
  misc_feature 1..1574: function = circular polyribonucleotide encoding turboGFP
gaaaatccgttgaccttaaacggtcgtgtgggttcaagtccctccacccccaattaggagactagaggacggtgagagtgaccagatgagataaacgcaatagcggaaaaactttaaacattaaaacccccctctccctccccccctaacgttactggccgaagccgcttggaataaggccggtgtgcgtttgtctatatgttattttccaccatattgccgtcttttggcaatgtgagggcccggaaacctggccctgtcttcttgacgagcattcctaggggtctttcccctctcgccaaaggaatgcaaggtctgttgaatgtcgtgaaggaagcagttcctctggaagcttcttgaagacaaacaacgtctgtagcgaccctttgcaggcagcggaaccccccacctggcgacaggtgcctctgcggccaaaagccacgtgtataagatacacctgcaaaggcggcacaaccccagtgccacgttgtgagttggatagttgtggaaagagtcaaatggctctcctcaagcgtattcaacaaggggctgaaggatgcccagaaggtaccccattgtatgggatctgatctggggcctcggtgcacatgctttacatgtgtttagtcgaggttaaaaaacgtctaggccccccgaaccacggggacgtggttttcctttgaaaaacacgatgataatatggccacaaccatggagagcgacgagagcggcctgcccgccatggagatcgagtgccgcatcaccggcaccctgaacggcgtggagttcgagctggtgggcggcggagagggcacccccgagcagggccgcatgaccaacaagatgaagagcaccaaaggcgccctgaccttcagcccctacctgctgagccacgtgatgggctacggcttctaccacttcggcacctaccccagcggctacgagaaccccttcctgcacgccatcaacaacggcggctacaccaacacccgcatcgagaagtacgaggacggcggcgtgctgcacgtgagcttcagctaccgctacgaggccggccgcgtgatcggcgacttcaaggtgatgggcaccggcttccccgaggacagcgtgatcttcaccgacaagatcatccgcagcaacgccaccgtggagcacctgcaccccatgggcgataacgatctggatggcagcttcacccgcaccttcagcctgcgcgacggcggctactacagctccgtggtggacagccacatgcacttcaagagcgccatccaccccagcatcctgcagaacgggggccccatgttcgccttccgccgcgtggaggaggatcacagcaacaccgagctgggcatcgtggagtaccagcacgccttcaagaccccggatgcagatgccggtgaagaataatctagactcgagctgtaatttacaaaaaacaaaacggcttaaatgcctaatataatatacgtctagactcccaatctcggactctaagcctgaagagaaaagcaagttcttgtaagtttaaccataaatttgccagccacggcaagctagacgctacggactta